European Patent Specification EP 3 587 593 B1, published September 27, 2023. Title: COMPOSITIONS, METHODS AND KITS TO DETECT HERPES SIMPLEX VIRUS NUCLEIC ACIDS. Applicant: Gen-Probe Incorporated Getman, Damon Chen, Wendy Aiyer, Aparna. Application To Be Assigned. The sequence listing filed with the application follows.

SEQUENCE LISTING (25 sequences)

SEQ ID NO: 1 - DNA, 480 bp, human herpesvirus 1
  ref <308>: X14112.1  GI:1944536
  ref <309>: 1997-04-18
  ref <313>: (142744)..(143223)
atggatccggctttgagatcttatcaccaacggctccgtctgtatacccccgtagcgatgggcatcaatctcgccgccagctcacaacctttggatccggaaggcccgatcgccgttactcccaggcctccgattcgtccgtcttctggtaaggcgccccatcccgaggccccacgtcggtcgccgaactgggcgaccgccggcgaggtggacgtcggagacgagctaatcgcgatttccgacgaacgcggacccccccgacatgaccgcccgcccctcgccacgtcgaccgcgccctcgccacacccgcgacccccgggctacacggccgttgtctccccgatggccctccaggctgtcgacgccccctccctgtttgtcgcctggctggccgctcggtggctccggggggcttccggcctgggggccgtcctgtgtgggattgcgtggtatgtgacgtcaattgcccgaggcgcataa

SEQ ID NO: 2 - DNA, 441 bp, Human herpesvirus 2
  ref <308>: NC_001798.1  GI:9629267
  ref <309>: 2000-08-01
  ref <313>: (145329)..(145769)
atggatccggctttgagatcttatcaccaacggctccgtctgtatacccccatagcgaggggcgtaaatctcgccgcccgctcaccacctttggttcgggaagcccgggccgtcgtcactcccaggcctcctatccgtccgtcctctggtaaggcgtcttccgacgacgcggacgtcggcgatgaactgattgccatcgcggacgcacgcggggacccgccagagaccctgccccccggcgcgggcggcgccgcgcccgcgtgccgcagaccacctcgcggcggctcccccgcggcctttcccgtggccctccacgccgtggacgccccctcccaattcgtcacctggctcgccgtgcgctggctgcggggggcggtgggtctcggggccgtcctgtgcgggattgcgttttacgtgacgtcaatcgcccgaggcgcataa

SEQ ID NO: 3 - DNA, 58 bp, Artificial Sequence
  synthetic oligomer
  misc_feature (26)..(58): polyd(T) and/or a poly(A) tail
atgcgcctcgggcgattgacgtcactttaaaaaaaaaaaaaaaaaaaaaaaaaaaaaa

SEQ ID NO: 4 - DNA, 25 bp, Artificial Sequence
  Synthetic Oligomer
atgcgcctcgggcgattgacgtcac

SEQ ID NO: 5 - DNA, 57 bp, Artificial Sequence
  Synthetic Oligomer
  misc_feature (25)..(57): polyd(T) and/or a poly(A) tail
ggtatacagacggagccgttggtgtttaaaaaaaaaaaaaaaaaaaaaaaaaaaaaa

SEQ ID NO: 6 - DNA, 24 bp, Artificial Sequence
  Synthetic Oligomer
ggtatacagacggagccgttggtg

SEQ ID NO: 7 - DNA, 20 bp, Artificial Sequence
  Synthetic Oligomer
aggcctccgattcgtccgtc

SEQ ID NO: 8 - DNA, 21 bp, Artificial Sequence
  Synthetic Oligomer
cgtccgtcttctggtaaggcg

SEQ ID NO: 9 - DNA, 50 bp, Artificial Sequence
  Synthetic Oligomer
  promoter (1)..(27)
aatttaatacgactcactatagggagaattagctcgtctccgacgtccac

SEQ ID NO: 10 - DNA, 23 bp, Artificial Sequence
  Synthetic Oligomer
attagctcgtctccgacgtccac

SEQ ID NO: 11 - DNA, 18 bp, Artificial Sequence
  Synthetic Oligomer
tcgtcactcccaggcctc

SEQ ID NO: 12 - DNA, 21 bp, Artificial Sequence
  Synthetic Oligomer
aggcctcctatccgtccgtcc

SEQ ID NO: 13 - DNA, 18 bp, Artificial Sequence
  Synthetic Oligomer
cacgtcggtcgccgaact

SEQ ID NO: 14 - DNA, 20 bp, Artificial Sequence
  Synthetic Oligomer
tcggtcgccgaactgggcga

SEQ ID NO: 15 - DNA, 49 bp, Artificial Sequence
  Synthetic Oligomer
  promoter (1)..(27)
aatttaatacgactcactatagggagacaatcagttcatcgccgacgtc

SEQ ID NO: 16 - DNA, 22 bp, Artificial Sequence
  Synthetic Oligomer
caatcagttcatcgccgacgtc

SEQ ID NO: 17 - DNA, 48 bp, Artificial Sequence
  Synthetic Oligomer
  promoter (1)..(27)
aatttaatacgactcactatagggagagcgatggcaatcagttcatcg

SEQ ID NO: 18 - DNA, 21 bp, Artificial Sequence
  Synthetic Oligomer
gcgatggcaatcagttcatcg

SEQ ID NO: 19 - DNA, 20 bp, Artificial Sequence
  Synthetic Oligomer
ggtaaggcgtcttccgacga

SEQ ID NO: 20 - DNA, 20 bp, Artificial Sequence
  Synthetic Oligomer
taaggcgtcttccgacgacg

SEQ ID NO: 21 - DNA, 47 bp, Artificial Sequence
  Synthetic oligomer
  promoter (1)..(27)
aatttaatacgactcactatagggagatcgtctccgacgtccacctc

SEQ ID NO: 22 - DNA, 20 bp, Artificial Sequence
  Synthetic Oligomer
tcgtctccgacgtccacctc

SEQ ID NO: 23 - DNA, 2555 bp, Herpes Simplex Virus 1
  ref <308>: NC_001806.1
  ref <309>: 2000-08-01
  ref <313>: (141139)..(143693)
catttaaggcgttgttgtgttgactttgcctcttctggcgggttggtgcggtgctgtttgttgggctcccattttacccgaagatcggctgctatccccgggacatggatcgcggggcggtggtggggtttcttctcggtgtttgtgttgtatcgtgcttggcgggaacgcccaaaacgtcctggagacgggtgagtgtcggcgaggacgtttcgttgcttccagctccggggcctacggggcgcggcccgacccagaaactactatgggccgtggaacccctggatgggtgcggccccttacacccgtcgtgggtctcgctgatgccccccaagcaggtgcccgagacggtcgtggatgcggcgtgcatgcgcgctccggtcccgctggcgatggcgtacgcccccccggccccatctgcgaccgggggtctacgaacggacttcgtgtggcaggagcgcgcggccgtggttaaccggagtctggttattcacggggtccgagagacggacagcggcctgtataccctgtccgtgggcgacataaaggacccggctcgccaagtggcctcggtggtcctggtggtgcaaccggccccagttccgaccccacccccgaccccagccgattacgacgaggatgacaatgacgagggcgaggacgaaagtctcgccggcactcccgccagcgggaccccccggctcccgcctccccccgcccccccgaggtcttggcccagcgcccccgaagtctcacatgtgcgtggggtgaccgtgcgtatggagactccggaagctatcctgttttcccccggggagacgttcagcacgaacgtctccatccatgccatcgcccacgacgaccagacctactccatggacgtcgtctggttgaggttcgacgtgccgacctcgtgtgccgagatgcgaatatacgaatcgtgtctgtatcacccgcagctcccagaatgtctgtccccggccgacgcgccgtgcgccgcgagtacgtggacgtctcgcctggccgtccgcagctacgcggggtgttccagaacaaaccccccaccgcgctgttcggccgaggctcacatggagcccgtcccggggctggcgtggcaggcggcctccgtcaatctggagttccgggacgcgtccccacaacactccggcctgtatctgtgtgtggtgtacgtcaacgaccatattcacgcctggggccacattaccatcagcaccgcggcgcagtaccggaacgcggtggtggaacagcccctcccacagcgcggcgcggatttggccgagcccacccacccgcacgtcggggcccctccccacgcgcccccaacccacggcgccctgcggttaggggcggtgatgggggccgccctgctgctgtctgcactggggttgtcggtgtgggcgtgtatgacctgttggcgcaggcgtgcctggcgggcggttaaaagcagggcctcgggtaaggggcccacgtacattcgcgtggccgacagcgagctgtacgcggactggagctcggacagcgagggagaacgcgaccaggtcccgtggctggcccccccggagagacccgactctccctccaccaatggatccggctttgagatcttatcaccaacggctccgtctgtatacccccgtagcgatgggcatcaatctcgccgccagctcacaacctttggatccggaaggcccgatcgccgttactcccaggcctccgattcgtccgtcttctggtaaggcgccccatcccgaggccccacgtcggtcgccgaactgggcgaccgccggcgaggtggacgtcggagacgagctaatcgcgatttccgacgaacgcggacccccccgacatgaccgcccgcccctcgccacgtcgaccgcgccctcgccacacccgcgacccccgggctacacggccgttgtctccccgatggccctccaggctgtcgacgccccctccctgtttgtcgcctggctggccgctcggtggctccggggggcttccggcctgggggccgtcctgtgtgggattgcgtggtatgtgacgtcaattgcccgaggcgcataaagggccggtggtccgcctagccgcagcaaattaaaaatcgtgagtcacagcgaccgcaacttcccacccggagctttcttccggcctcgatgacgtcccggctctccgatcccaactcctcagcgcgatccgacatgtccgtgccgctttatcccacggcctcgccagtttcggtcgaagcctactactcggaaagcgaagacgaggcggccaacgacttcctcgtacgcatgggccgccaacagtcggtattaaggcgtcgacgcagacgcacccgctgcgtcggcatggtgatcgcctgtctcctcgtggccgttctgtcgggcggatttggggcgctcctgatgtggctgctccgctaaaagaccgcatcgacacgcgcgtccttcttgtcgtctctcttcccccccatcaccccgcaatttgcacccagcctttaactacattaaattgggttcgattggcaatgt

SEQ ID NO: 24 - DNA, 2371 bp, Herpes Simplex Virus 2
  ref <308>: NC_001798.1
  ref <309>: 2000-08-01
  ref <313>: (143843)..(146213)
atggctcgcggggccgggttggtgttttttgttggagtttgggtcgtatcgtgcctggcggcagcacccagaacgtcctggaaacgggtaacctcgggcgaggacgtggtgttgcttccggcgcccgcggaacgcacccgggcccacaaactactgtgggccgcggaacccctggatgcctgcggtcccctgcgcccgtcgtgggtggcgctgtggcccccccgacgggtgctcgagacggtcgtggatgcggcgtgcatgcgcgccccggaaccgctcgccatagcatacagtcccccgttccccgcgggcgacgagggactgtattcggagttggcgtggcgcgatcgcgtagccgtggtcaacgagagtctggtcatctacggggccctggagacggacagcggtctgtacaccctgtccgtggtcggcctaagcgacgaggcgcgccaagtggcgtcggtggttctggtcgtggagcccgcccctgtgccgaccccgacccccgacgactacgacgaagaagacgacgcgggcgtgacgaacgcacgccggtcagcgttccccccccaaccccccccccgtcgtccccccgtcgcccccccgacgcaccctcgtgttatccccgaggtgtcccacgtgcgcggggtaacggtccatatggagaccctggaggccattctgtttgcccccggggagacgtttgggacgaacgtctccatccacgccattgcccacgacgacggtccgtacgccatggacgtcgtctggatgcggtttgacgtgccgtcctcgtgcgccgatatgcggatctacgaagcttgtctgtatcacccgcagcttccagagtgtctatctccggccgacgcgccgtgcgccgtaagttcctgggcgtaccgcctggcggtccgcagctacgccggctgttccaggactacgcccccgccgcgatgttttgccgaggctcgcatggaaccggtcccggggttggcgtggctggcctccaccgtcaatctggaattccagcacgcctccccccagcacgccggcctctacctgtgcgtggtgtacgtggacgatcatatccacgcctggggccacatgaccatcagcaccgcggcgcagtaccggaacgcggtggtggaacagcacctcccccagcgccagcccgagcccgtcgagcccacccgcccgcacgtgagagccccccatcccgcgccctccgcgcgcggcccgctgcgcctcggggcggtgctgggggcggccctgttgctggccgccctcgggctgtccgcgtgggcgtgcatgacctgctggcgcaggcgctcctggcgggcggttaaaagccgggcctcggcgacgggccccacttacattcgcgtggcggacagcgagctgtacgcggactggagttcggacagcgagggggagcgcgacgggtccctgtggcaggaccctccggagagacccgactctccctccacaaatggatccggctttgagatcttatcaccaacggctccgtctgtatacccccatagcgaggggcgtaaatctcgccgcccgctcaccacctttggttcgggaagcccgggccgtcgtcactcccaggcctcctatccgtccgtcctctggtaaggcgtcttccgacgacgcggacgtcggcgatgaactgattgccatcgcggacgcacgcggggacccgccagagaccctgccccccggcgcgggcggcgccgcgcccgcgtgccgcagaccacctcgcggcggctcccccgcggcctttcccgtggccctccacgccgtggacgccccctcccaattcgtcacctggctcgccgtgcgctggctgcggggggcggtgggtctcggggccgtcctgtgcgggattgcgttttacgtgacgtcaatcgcccgaggcgcataaaggtccggcggccaccccgccgcagctcataaaaatcgtgagtcacggcaaccccaccttcgcctccgccctccgccagcgcccttccgcgtccgcgatgacctcccggcccgccgaccaagactcggtgcgttccagcgcgtcggtgccgctttaccccgcggcctcgcccgtcccggcagaagcctactactcggaaagcgaagacgaggccgccaacgacttcctcgtgcgcatgggccgccagcagtcggtcctaaggcgccgacggcggcgcacgcggtgcgtcgggctggttatcgcctgtctcgtcgtggccctcctatctggagggttcggggcacttttggtgtggctgctccgctaaatgacgcctcgatgtatggcgccttcttcgcccccacccctcgccgcgacccacgtccgtatgttaattgcaataaa

SEQ ID NO: 25 - DNA, 950 bp, Herpes Simplex Virus 1
  ref <308>: NC_001806.1
  ref <309>: 2000-08-01
  ref <313>: (142744)..(143693)
atggatccggctttgagatcttatcaccaacggctccgtctgtatacccccgtagcgatgggcatcaatctcgccgccagctcacaacctttggatccggaaggcccgatcgccgttactcccaggcctccgattcgtccgtcttctggtaaggcgccccatcccgaggccccacgtcggtcgccgaactgggcgaccgccggcgaggtggacgtcggagacgagctaatcgcgatttccgacgaacgcggacccccccgacatgaccgcccgcccctcgccacgtcgaccgcgccctcgccacacccgcgacccccgggctacacggccgttgtctccccgatggccctccaggctgtcgacgccccctccctgtttgtcgcctggctggccgctcggtggctccggggggcttccggcctgggggccgtcctgtgtgggattgcgtggtatgtgacgtcaattgcccgaggcgcataaagggccggtggtccgcctagccgcagcaaattaaaaatcgtgagtcacagcgaccgcaacttcccacccggagctttcttccggcctcgatgacgtcccggctctccgatcccaactcctcagcgcgatccgacatgtccgtgccgctttatcccacggcctcgccagtttcggtcgaagcctactactcggaaagcgaagacgaggcggccaacgacttcctcgtacgcatgggccgccaacagtcggtattaaggcgtcgacgcagacgcacccgctgcgtcggcatggtgatcgcctgtctcctcgtggccgttctgtcgggcggatttggggcgctcctgatgtggctgctccgctaaaagaccgcatcgacacgcgcgtccttcttgtcgtctctcttcccccccatcaccccgcaatttgcacccagcctttaactacattaaattgggttcgattggcaatgt